European Patent Application EP 4 796 121 A2, published August 26, 2026. Title: Combination of RNA and immune checkpoint inhibitors. Applicant: CureVac SE. Application EP. The sequence listing filed with the application follows.

SEQUENCE LISTING (35 sequences)

SEQ ID NO: 1 - RNA, 1480 nt, synthetic construct
  misc_feature 1..1480: note = 5T4 (GC)-muag-A64-C30-HistoneSL
  source 1..1480: mol_type = other RNA
gggagaaagcttaccatgcccggcgggtgcagccggggcccggccgccggggacggccgcctgcggctcgcgcgcctggccctggtgctcctggggtgggtctccagctccagccccacctccagcgcctccagcttctccagctccgcccccttcctggccagcgcggtgtccgcccagcccccgctccccgaccagtgccccgccctgtgcgagtgcagcgaggccgcgcggaccgtgaagtgcgtcaaccgcaacctgacggaggtgcccaccgacctcccggcctacgtgcggaacctgttcctgaccggcaaccagctcgccgtcctgcccgccggcgccttcgcgcgccggccgcccctggccgagctcgccgccctgaacctgtccgggagccgcctcgacgaggtgcgggccggcgcgttcgagcacctgccgtccctgcgccagctcgacctgagccacaaccccctggccgacctctcccccttcgccttcagcgggagcaacgcctccgtgagcgccccctccccgctggtcgagctgatcctcaaccacatcgtgccccccgaggacgagcggcagaaccgcagcttcgagggcatggtggtcgcggccctgctggccgggcgggccctccagggcctgcgccggctggagctcgcctccaaccacttcctgtacctgccccgcgacgtgctcgcgcagctgccgagcctgcggcacctcgacctgtccaacaacagcctggtgtccctcacctacgtcagcttccgcaacctgacgcacctggagtccctccacctggaggacaacgccctgaaggtgctgcacaacggcaccctcgccgagctgcaggggctgccccacatccgggtgttcctcgacaacaacccctgggtctgcgactgccacatggccgacatggtgacctggctgaaggagaccgaggtggtccagggcaaggaccgcctgacgtgcgcgtaccccgagaagatgcggaaccgggtgctcctggagctgaacagcgccgacctcgactgcgacccgatcctgcccccctccctgcagaccagctacgtgttcctcgggatcgtcctggccctgatcggcgccatcttcctcctggtgctgtacctcaaccgcaagggcatcaagaagtggatgcacaacatccgggacgcctgccgcgaccacatggaggggtaccactaccggtacgagatcaacgcggacccccgcctgaccaacctgtccagcaactccgacgtctgaccactagttataagactgactagcccgatgggcctcccaacgggccctcctcccctccttgcaccgagattaataaaaaaaaaaaaaaaaaaaaaaaaaaaaaaaaaaaaaaaaaaaaaaaaaaaaaaaaaaaaaaaatgcatcccccccccccccccccccccccccccccccaaaggctcttttcagagccaccagaatt

SEQ ID NO: 2 - RNA, 646 nt, synthetic construct
  misc_feature 1..646: note = Survivin (GC)-muag-A64-C30-HistoneSL
  source 1..646: mol_type = other RNA
gggagaaagcttaccatgggcgcccccaccctgccgccggcctggcagccgttcctcaaggaccaccgcatctcgaccttcaagaactggccgttcctggagggctgcgcgtgcaccccggagcggatggccgaggccggcttcatccactgccccaccgagaacgagccggacctggcccagtgcttcttctgcttcaaggagctggagggctgggagccggacgacgacccgatcgaggagcacaagaagcacagcagcggctgcgccttcctgagcgtgaagaagcagttcgaggagctgacgctcggggagttcctgaagctggaccgggagcgggccaagaacaagatcgcgaaggagaccaacaacaagaagaaggagttcgaggagaccgccaagaaggtgcggcgggccatcgagcagctggccgccatggactgaccactagttataagactgactagcccgatgggcctcccaacgggccctcctcccctccttgcaccgagattaataaaaaaaaaaaaaaaaaaaaaaaaaaaaaaaaaaaaaaaaaaaaaaaaaaaaaaaaaaaaaaaatgcatcccccccccccccccccccccccccccccccaaaggctcttttcagagccaccagaatt

SEQ ID NO: 3 - RNA, 760 nt, synthetic construct
  misc_feature 1..760: note = NY-ESO-1 (GC)-muag-A64-C30-histone SL
  source 1..760: mol_type = other RNA
gggagaaagcttaccatgcaggccgagggccgcggcaccggcggctcgaccggcgacgccgacgggcccggcggcccgggcatcccggacggcccgggcgggaacgcgggcggcccgggcgaggccggcgccaccggcgggcggggcccgcggggcgccggcgccgcccgggcgagcggccccggcgggggcgccccgcggggcccgcacggcggcgccgccagcggcctgaacgggtgctgccggtgcggcgcccgcggcccggagagccggctcctggagttctacctggccatgccgttcgcgaccccgatggaggccgagctggcccggcggagcctggcccaggacgccccgccgctgcccgtgccgggcgtgctcctgaaggagttcacggtgagcggcaacatcctgaccatccggctgaccgccgcggaccaccggcagctgcagctgtcgatcagcagctgcctccagcagctgagcctgctgatgtggatcacccagtgcttcctgccggtgttcctggcccagccgcccagcggccagcgccggtgaccactagttataagactgactagcccgatgggcctcccaacgggccctcctcccctccttgcaccgagattaataaaaaaaaaaaaaaaaaaaaaaaaaaaaaaaaaaaaaaaaaaaaaaaaaaaaaaaaaaaaaaaatgcatcccccccccccccccccccccccccccccccaaaggctcttttcagagccaccagaatt

SEQ ID NO: 4 - RNA, 1813 nt, synthetic construct
  misc_feature 1..1813: note = MAGE-C1 (aa 613-1142) (GC)-muag-A64-C30-histoneSL
  source 1..1813: mol_type = other RNA
gggagaaagcttaccatgcagtccccgctgcagggcgaggagttccagagctccctgcagagccccgtgtccatctgcagctccagcaccccctccagcctcccgcagagcttccccgagtccagccagtccccccccgagggcccggtccagagccccctgcactccccgcagagccccccggaggggatgcactcccagagccccctgcagtcccccgagagcgcccccgagggcgaggactccctcagcccgctgcagatcccccagtccccgctggagggggaggacagcctctccagcctgcacttcccccagtccccgcccgagtgggaggacagcctgagccccctccacttcccccagttcccgccccagggcgaggacttccagtccagcctgcagtcccccgtgagcatctgctccagctccacgagcctgtccctcccccagagcttcccggagtccccccagagcccgcccgaggggccggcgcagtcccccctgcagcgccccgtgagctccttcttcagctacaccctggcctccctcctgcagagctcccacgagagcccgcagagcccgcccgagggccccgcccagtccccgctgcagagccccgtctccagcttcccctccagcacctccagctccctcagccagtccagccccgtgtccagcttcccgtccagcacctccagctccctgagcaagagctcccccgagagccccctgcagtcccccgtgatcagcttctccagctccacgagcctctccccgttcagcgaggagtccagctcccccgtcgacgagtacaccagctccagcgacaccctgctggagtccgacagcctcaccgactccgagagcctgatcgagagcgagcccctgttcacctacacgctcgacgagaaggtggacgagctggcccggttcctgctcctgaagtaccaggtgaagcagcccatcaccaaggccgagatgctgaccaacgtcatctcccgctacaccggctacttcccggtgatcttccggaaggcgcgcgagttcatcgagatcctcttcgggatcagcctgcgggaggtggaccccgacgactcctacgtcttcgtgaacacgctggacctcaccagcgagggctgcctgtccgacgagcaggggatgagccagaaccgcctgctcatcctgatcctgtccatcatcttcatcaagggcacctacgccagcgaggaggtcatctgggacgtgctctccgggatcggcgtgcgggccggccgcgagcacttcgccttcggggagccccgggagctgctgaccaaggtctgggtgcaggagcactacctcgagtaccgcgaggtgcccaacagctccccgccccggtacgagttcctgtggggcccccgcgcccacagcgaggtcatcaagcggaaggtggtggagttcctggcgatgctcaagaacacggtccccatcaccttcccgtccagctacaaggacgccctgaaggacgtggaggagcgggcccaggccatcatcgacaccaccgacgactccacggccaccgagagcgcgtccagctccgtgatgagccccagcttctccagcgagtgaccactagttataagactgactagcccgatgggcctcccaacgggccctcctcccctccttgcaccgagattaataaaaaaaaaaaaaaaaaaaaaaaaaaaaaaaaaaaaaaaaaaaaaaaaaaaaaaaaaaaaaaaatgcatcccccccccccccccccccccccccccccccaaaggctcttttcagagccaccagaatt

SEQ ID NO: 5 - RNA, 1339 nt, synthetic construct
  misc_feature 1..1339: note = MAGE-C2 (GC)-muag-A64-C30-histoneSL
  source 1..1339: mol_type = other RNA
gggagaaagcttaccatgcccccggtgcccggcgtccccttccggaacgtggacaacgacagccccacctccgtggagctggaggactgggtcgacgcccagcacccgaccgacgaggaggaggaggaggccagctccgcgagctccacgctctacctggtgttcagcccctccagcttctccaccagctccagcctgatcctcgggggccccgaggaggaggaggtgccctccggggtcatcccgaacctgaccgagagcatcccctccagccccccgcagggcccgccccaggggccctcccagagccccctgtccagctgctgcagctccttcagctggtccagcttctccgaggagagctccagccagaagggcgaggacaccggcacgtgccaggggctcccggactccgagagctccttcacctacaccctggacgagaaggtggccgagctggtggagttcctcctgctgaagtacgaggccgaggagcccgtcaccgaggccgagatgctcatgatcgtgatcaagtacaaggactacttccccgtgatcctgaagcgcgcccgggagttcatggagctgctcttcggcctggcgctgatcgaggtcgggcccgaccacttctgcgtgttcgccaacacggtgggcctcaccgacgaggggagcgacgacgagggcatgccggagaactccctgctgatcatcatcctcagcgtcatcttcatcaagggcaactgcgcctccgaggaggtgatctgggaggtgctgaacgccgtcggggtgtacgcgggccgcgagcacttcgtgtacggggagccccgggagctgctcaccaaggtctgggtgcagggccactacctggagtaccgcgaggtgccgcacagctcccccccgtactacgagttcctgtggggcccccgggcccacagcgagtccatcaagaagaaggtcctcgagttcctggccaagctgaacaacaccgtgcccagcagcttcccctcctggtacaaggacgccctcaaggacgtcgaggagcgcgtgcaggccacgatcgacaccgcggacgacgccaccgtgatggccagcgagtccctgagcgtcatgtccagcaacgtgtccttcagcgagtgaccactagttataagactgactagcccgatgggcctcccaacgggccctcctcccctccttgcaccgagattaataaaaaaaaaaaaaaaaaaaaaaaaaaaaaaaaaaaaaaaaaaaaaaaaaaaaaaaaaaaaaaaatgcatcccccccccccccccccccccccccccccccaaaggctcttttcagagccaccagaatt

SEQ ID NO: 6 - RNA, 1885 nt, synthetic construct
  misc_feature 1..1885: note = MUC1 5 VNTR (GC)-muag-A64-C30-histoneSL
  source 1..1885: mol_type = other RNA
gggagaaagcttaccatgacccccggcacccagagcccgttcttcctgctcctgctgctcacggtgctgaccgtcgtgaccgggtccggccacgccagctccacccccgggggcgagaaggagacgagcgccacccagcggtccagcgtgccctccagcaccgagaagaacgcggtctccatgaccagctccgtgctgagctcccacagccccgggtccggcagctccacgacccagggccaggacgtgaccctcgccccggccaccgagcccgccagcgggtccgccgcgacgtggggccaggacgtcaccagcgtgcccgtgacccgccccgccctggggagcaccacgccgcccgcccacgacgtcacctccgcccccgacaacaagcccgcgccgggcagcaccgccccccccgcccacggggtgacctccgcccccgacacgcggccggcccccggcagcaccgcgccccccgcccacggcgtgacctccgccccggacacccgccccgcccccgggagcacggccccgccggcgcacggcgtcacctccgcccccgacacccggcccgcccccgggagcaccgccccgcccgcccacggcgtgacgtccgcgcccgacacccgcccggcccccggcagcaccgccccccccgcccacggggtgacctccgccccggacacgcggcccgcgcccggcagcaccgccccgccggcccacggggtcacctccgcgcccgacaaccgccccgccctggggagcaccgccccgcccgtgcacaacgtgacctccgccagcggctccgcgagcgggtccgccagcaccctcgtccacaacggcacgtccgcccgggccaccaccacccccgccagcaagtccacgcccttcagcatcccgtcccaccacagcgacacccccaccaccctggcgtcccacagcacgaagaccgacgcctccagcacccaccactccagcgtgcccccgctgaccagctccaaccacagcacgtccccgcagctcagcaccggggtgtccttcttcttcctgagcttccacatctccaacctgcagttcaacagctccctcgaggaccccagcaccgactactaccaggagctgcagcgggacatctccgagatgttcctgcagatctacaagcagggcggcttcctcgggctgagcaacatcaagttccgccccggctccgtcgtggtgcagctgaccctcgccttccgggaggggacgatcaacgtccacgacgtggagacccagttcaaccagtacaagaccgaggccgccagccgctacaacctgaccatctccgacgtgagcgtctccgacgtgcccttcccgttcagcgcgcagtccggcgccggcgtgcccgggtggggcatcgccctgctcgtcctggtgtgcgtgctggtcgccctcgccatcgtgtacctgatcgcgctggccgtgtgccagtgccggcgcaagaactacgggcagctcgacatcttccccgcccgggacacgtaccacccgatgagcgagtacccgacctaccacacccacggccgctacgtcccccccagctccaccgaccggagcccctacgagaaggtgtccgccgggaacggcggcagctccctgagctacaccaacccggcggtggccgccgcctccgccaacctgtgaccactagttataagactgactagcccgatgggcctcccaacgggccctcctcccctccttgcaccgagattaataaaaaaaaaaaaaaaaaaaaaaaaaaaaaaaaaaaaaaaaaaaaaaaaaaaaaaaaaaaaaaaatgcatcccccccccccccccccccccccccccccccaaaggctcttttcagagccaccagaatt

SEQ ID NO: 7 - RNA, 13 nt, synthetic construct
  misc_feature 1..13: note = Kozak sequence
  source 1..13: mol_type = other RNA
gccgccaccatgg

SEQ ID NO: 8 - DNA, 186 bp, human
  source 1..186: mol_type = other DNA
catcacatttaaaagcatctcagcctaccatgagaataagagaaagaaaatgaagatcaaaagcttattcatctgtttttctttttcgttggtgtaaagccaacaccctgtctaaaaaacataaatttctttaatcattttgcctcttttctctgtgcttcaattaataaaaaatggaaagaatct

SEQ ID NO: 9 - DNA, 186 bp, human
  source 1..186: mol_type = other DNA
catcacatttaaaagcatctcagcctaccatgagaataagagaaagaaaatgaagatcaatagcttattcatctctttttctttttcgttggtgtaaagccaacaccctgtctaaaaaacataaatttctttaatcattttgcctcttttctctgtgcttcaattaataaaaaatggaaagaacct

SEQ ID NO: 10 - DNA, 110 bp, human
  source 1..110: mol_type = other DNA
gctggagcctcggtggccatgcttcttgccccttgggcctccccccagcccctcctccccttcctgcacccgtacccccgtggtctttgaataaagtctgagtgggcggc

SEQ ID NO: 11 - DNA, 108 bp, human
  source 1..108: mol_type = other DNA
gctggagcctcggtagccgttcctcctgcccgctgggcctcccaacgggccctcctcccctccttgcaccggcccttcctggtctttgaataaagtctgagtgggcag

SEQ ID NO: 12 - DNA, 132 bp, human
  source 1..132: mol_type = other DNA
gctcgctttcttgctgtccaatttctattaaaggttcctttgttccctaagtccaactactaaactgggggatattatgaagggccttgagcatctggattctgcctaataaaaaacatttattttcattgc

SEQ ID NO: 13 - DNA, 44 bp, synthetic construct
  misc_feature 1..44: note = Center, alpha-complex-binding portion of the 3 UTR of an alpha-globin gene
  source 1..44: mol_type = other DNA
gcccgatgggcctcccaacgggccctcctcccctccttgcaccg

SEQ ID NO: 14 - DNA, 75 bp, synthetic construct
  misc_feature 1..75: note = 5'UTR of human ATP5A1 lacking the 5' terminal oligopyrimidine tract
  source 1..75: mol_type = other DNA
gcggctcggccattttgtcccagtcagtccggaggctgcggctgcagaagtaccgcctgcggagtaactgcaaag

SEQ ID NO: 15 - DNA, 42 bp, synthetic construct
  misc_feature 1..42: note = 5-UTR of human ribosomal protein Large 32 lacking the 5 terminal oligopyrimidine tract
  source 1..42: mol_type = other DNA
ggcgctgcctacggaggtggcagccatctccttctcggcatc

SEQ ID NO: 16 - DNA, 62 bp, synthetic construct
  misc_feature 1..62: note = 5'UTR of human HSD17B4 lacking the 5' terminal oligopyrimidine tract
  source 1..62: mol_type = other DNA
gtcccgcagtcggcgtccagcggctctgcttgttcgtgtgtgtgtcgttgcaggccttattc

SEQ ID NO: 17 - DNA, 24 bp, synthetic construct
  misc_feature 1..24: note = histone stem loop
  source 1..24: mol_type = other DNA
caaaggctcttttcagagccacca

SEQ ID NO: 18 - RNA, 24 nt, synthetic construct
  misc_feature 1..24: note = histone stem loop
  source 1..24: mol_type = other RNA
caaaggctcttttcagagccacca

SEQ ID NO: 19 - protein, 447 aa, synthetic construct
  REGION 1..447: note = Pembrolizumab_HeavyChain1__Any
QVQLVQSGVEVKKPGASVKVSCKASGYTFTNYYMYWVRQAPGQGLEWMGGINPSNGGTNFNEKFKNRVTLTTDSSTTTAYMELKSLQFDDTAVYYCARRDYRFDMGFDYWGQGTTVTVSSASTKGPSVFPLAPCSRSTSESTAALGCLVKDYFPEPVTVSWNSGALTSGVHTFPAVLQSSGLYSLSSVVTVPSSSLGTKTYTCNVDHKPSNTKVDKRVESKYGPPCPPCPAPEFLGGPSVFLFPPKPKDTLMISRTPEVTCVVVDVSQEDPEVQFNWYVDGVEVHNAKTKPREEQFNSTYRVVSVLTVLHQDWLNGKEYKCKVSNKGLPSSIEKTISKAKGQPREPQVYTLPPSQEEMTKNQVSLTCLVKGFYPSDIAVEWESNGQPENNYKTTPPVLDSDGSFFLYSRLTVDKSRWQEGNVFSCSVMHEALHNHYTQKSLSLSLGK

SEQ ID NO: 20 - protein, 218 aa, synthetic construct
  REGION 1..218: note = Pembrolizumab_LightChain1__Any
EIVLTQSPATLSLSPGERATLSCRASKGVSTSGYSYLHWYQQKPGQAPRLLIYLASYLESGVPARFSGSGSGTDFTLTISSLEPEDFAVYYCQHSRDLPLTFGGGTKVEIKRTVAAPSVFIFPPSDEQLKSGTASVVCLLNNFYPREAKVQWKVDNALQSGNSQESVTEQDSKDSTYSLSSTLTLSKADYEKHKVYACEVTHQGLSSPVTKSFNRGEC

SEQ ID NO: 21 - protein, 440 aa, synthetic construct
  REGION 1..440: note = Nivolumab_HeavyChain1__Any
QVQLVESGGGVVQPGRSLRLDCKASGITFSNSGMHWVRQAPGKGLEWVAVIWYDGSKRYYADSVKGRFTISRDNSKNTLFLQMNSLRAEDTAVYYCATNDDYWGQGTLVTVSSASTKGPSVFPLAPCSRSTSESTAALGCLVKDYFPEPVTVSWNSGALTSGVHTFPAVLQSSGLYSLSSVVTVPSSSLGTKTYTCNVDHKPSNTKVDKRVESKYGPPCPPCPAPEFLGGPSVFLFPPKPKDTLMISRTPEVTCVVVDVSQEDPEVQFNWYVDGVEVHNAKTKPREEQFNSTYRVVSVLTVLHQDWLNGKEYKCKVSNKGLPSSIEKTISKAKGQPREPQVYTLPPSQEEMTKNQVSLTCLVKGFYPSDIAVEWESNGQPENNYKTTPPVLDSDGSFFLYSRLTVDKSRWQEGNVFSCSVMHEALHNHYTQKSLSLSLGK

SEQ ID NO: 22 - protein, 214 aa, synthetic construct
  REGION 1..214: note = Nivolumab_LightChain1__Any
EIVLTQSPATLSLSPGERATLSCRASQSVSSYLAWYQQKPGQAPRLLIYDASNRATGIPARFSGSGSGTDFTLTISSLEPEDFAVYYCQQSSNWPRTFGQGTKVEIKRTVAAPSVFIFPPSDEQLKSGTASVVCLLNNFYPREAKVQWKVDNALQSGNSQESVTEQDSKDSTYSLSSTLTLSKADYEKHKVYACEVTHQGLSSPVTKSFNRGEC

SEQ ID NO: 23 - protein, 438 aa, synthetic construct
  REGION 1..438: note = REGN2810_HeavyChain1__Any
EVQLLESGGVLVQPGGSLRLSCAASGFTFSNFGTWVRQAPGKGLEWVSGISGGGRDTYFADSVKGRFTISRDNSKNTLYLQNSLKGEDTAVYYCVKWGNIYFDYWGQGTLVTVSSASTKGPSVFPLAPCSRSTSESTAALGCLVKDYFPEPVTVSWNSGALTSGVHTFPAVLQSSGLYSLSSVVTVPSSSLGTKTYTCNVDHKPSNTKVDKRVESKYGPPCPPCPAPEFLGGPSVFLFPPKPKDTLISRTPEVTCVVVDVSQEDPEVQFNWYVDGVEVHNAKTKPREEQFNSTYRVVSVLTVLHQDWLNGKEYKCKVSNKGLPSSIEKTISKAKGQPREPQVYTLPPSQEETKNQVSLTCLVKGFYPSDIAVEWESNGQPENNYKTTPPVLDSDGSFFLYSRLTVDKSRWQEGNVFSCSVHEALHNHYTQKSLSLSLG

SEQ ID NO: 24 - protein, 213 aa, synthetic construct
  REGION 1..213: note = REGN2810_LightChain1__Any
DIQTQSPSSLSASVGDSITITCRASLSINTFLNWYQQKPGKAPNLLIYAASSLHGGVPSRFSGSGSGTDFTLTIRTLQPEDFATYYCQQSSNTPFTFGPGTVVDFRRTVAAPSVFIFPPSDEQLKSGTASVVCLLNNFYPREAKVQWKVDNALQSGNSQESVTEQDSKDSTYSLSSTLTLSKADYEKHKVYACEVTHQGLSSPVTKSFNRGEC

SEQ ID NO: 25 - protein, 447 aa, synthetic construct
  REGION 1..447: note = Pidilizumab_HeavyChain1__Any
QVQLVQSGSELKKPGASVKISCKASGYTFTNYGMNWVRQAPGQGLQWMGWINTDSGESTYAEEFKGRFVFSLDTSVNTAYLQITSLTAEDTGMYFCVRVGYDALDYWGQGTLVTVSSASTKGPSVFPLAPSSKSTSGGTAALGCLVKDYFPEPVTVSWNSGALTSGVHTFPAVLQSSGLYSLSSVVTVPSSSLGTQTYICNVNHKPSNTKVDKRVEPKSCDKTHTCPPCPAPELLGGPSVFLFPPKPKDTLMISRTPEVTCVVVDVSHEDPEVKFNWYVDGVEVHNAKTKPREEQYNSTYRVVSVLTVLHQDWLNGKEYKCKVSNKALPAPIEKTISKAKGQPREPQVYTLPPSREEMTKNQVSLTCLVKGFYPSDIAVEWESNGQPENNYKTTPPVLDSDGSFFLYSKLTVDKSRWQQGNVFSCSVMHEALHNHYTQKSLSLSPGK

SEQ ID NO: 26 - protein, 213 aa, synthetic construct
  REGION 1..213: note = Pidilizumab_LightChain1__Any
EIVLTQSPSSLSASVGDRVTITCSARSSVSYMHWFQQKPGKAPKLWIYRTSNLASGVPSRFSGSGSGTSYCLTINSLQPEDFATYYCQQRSSFPLTFGGGTKLEIKRTVAAPSVFIFPPSDEQLKSGTASVVCLLNNFYPREAKVQWKVDNALQSGNSQESVTEQDSKDSTYSLSSTLTLSKADYEKHKVYACEVTHQGLSSPVTKSFNRGEC

SEQ ID NO: 27 - protein, 451 aa, synthetic construct
  REGION 1..451: note = Durvalumab_HeavyChain1__Any
EVQLVESGGGLVQPGGSLRLSCAASGFTFSRYWMSWVRQAPGKGLEWVANIKQDGSEKYYVDSVKGRFTISRDNAKNSLYLQMNSLRAEDTAVYYCAREGGWFGELAFDYWGQGTLVTVSSASTKGPSVFPLAPSSKSTSGGTAALGCLVKDYFPEPVTVSWNSGALTSGVHTFPAVLQSSGLYSLSSVVTVPSSSLGTQTYICNVNHKPSNTKVDKRVEPKSCDKTHTCPPCPAPEFEGGPSVFLFPPKPKDTLMISRTPEVTCVVVDVSHEDPEVKFNWYVDGVEVHNAKTKPREEQYNSTYRVVSVLTVLHQDWLNGKEYKCKVSNKALPASIEKTISKAKGQPREPQVYTLPPSREEMTKNQVSLTCLVKGFYPSDIAVEWESNGQPENNYKTTPPVLDSDGSFFLYSKLTVDKSRWQQGNVFSCSVMHEALHNHYTQKSLSLSPGK

SEQ ID NO: 28 - protein, 215 aa, synthetic construct
  REGION 1..215: note = Durvalumab_LightChain1__Any
EIVLTQSPGTLSLSPGERATLSCRASQRVSSSYLAWYQQKPGQAPRLLIYDASSRATGIPDRFSGSGSGTDFTLTISRLEPEDFAVYYCQQYGSLPWTFGQGTKVEIKRTVAAPSVFIFPPSDEQLKSGTASVVCLLNNFYPREAKVQWKVDNALQSGNSQESVTEQDSKDSTYSLSSTLTLSKADYEKHKVYACEVTHQGLSSPVTKSFNRGEC

SEQ ID NO: 29 - protein, 448 aa, synthetic construct
  REGION 1..448: note = Atezolizumab_HeavyChain1__Any
EVQLVESGGGLVQPGGSLRLSCAASGFTFSDSWIHWVRQAPGKGLEWVAWISPYGGSTYYADSVKGRFTISADTSKNTAYLQMNSLRAEDTAVYYCARRHWPGGFDYWGQGTLVTVSSASTKGPSVFPLAPSSKSTSGGTAALGCLVKDYFPEPVTVSWNSGALTSGVHTFPAVLQSSGLYSLSSVVTVPSSSLGTQTYICNVNHKPSNTKVDKKVEPKSCDKTHTCPPCPAPELLGGPSVFLFPPKPKDTLMISRTPEVTCVVVDVSHEDPEVKFNWYVDGVEVHNAKTKPREEQYASTYRVVSVLTVLHQDWLNGKEYKCKVSNKALPAPIEKTISKAKGQPREPQVYTLPPSREEMTKNQVSLTCLVKGFYPSDIAVEWESNGQPENNYKTTPPVLDSDGSFFLYSKLTVDKSRWQQGNVFSCSVMHEALHNHYTQKSLSLSPGK

SEQ ID NO: 30 - protein, 214 aa, synthetic construct
  REGION 1..214: note = Atezolizumab_LightChain1__Any
DIQMTQSPSSLSASVGDRVTITCRASQDVSTAVAWYQQKPGKAPKLLIYSASFLYSGVPSRFSGSGSGTDFTLTISSLQPEDFATYYCQQYLYHPATFGQGTKVEIKRTVAAPSVFIFPPSDEQLKSGTASVVCLLNNFYPREAKVQWKVDNALQSGNSQESVTEQDSKDSTYSLSSTLTLSKADYEKHKVYACEVTHQGLSSPVTKSFNRGEC

SEQ ID NO: 31 - protein, 450 aa, synthetic construct
  REGION 1..450: note = Avelumab_HeavyChain1__Any
EVQLLESGGGLVQPGGSLRLSCAASGFTFSSYIMMWVRQAPGKGLEWVSSIYPSGGITFYADTVKGRFTISRDNSKNTLYLQMNSLRAEDTAVYYCARIKLGTVTTVDYWGQGTLVTVSSASTKGPSVFPLAPSSKSTSGGTAALGCLVKDYFPEPVTVSWNSGALTSGVHTFPAVLQSSGLYSLSSVVTVPSSSLGTQTYICNVNHKPSNTKVDKKVEPKSCDKTHTCPPCPAPELLGGPSVFLFPPKPKDTLMISRTPEVTCVVVDVSHEDPEVKFNWYVDGVEVHNAKTKPREEQYNSTYRVVSVLTVLHQDWLNGKEYKCKVSNKALPAPIEKTISKAKGQPREPQVYTLPPSRDELTKNQVSLTCLVKGFYPSDIAVEWESNGQPENNYKTTPPVLDSDGSFFLYSKLTVDKSRWQQGNVFSCSVMHEALHNHYTQKSLSLSPGK

SEQ ID NO: 32 - protein, 216 aa, synthetic construct
  REGION 1..216: note = Avelumab_LightChain1__Any
QSALTQPASVSGSPGQSITISCTGTSSDVGGYNYVSWYQQHPGKAPKLMIYDVSNRPSGVSNRFSGSKSGNTASLTISGLQAEDEADYYCSSYTSSSTRVFGTGTKVTVLGQPKANPTVTLFPPSSEELQANKATLVCLISDFYPGAVTVAWKADGSPVKAGVETTKPSKQSNNKYAASSYLSLTPEQWKSHRSYSCQVTHEGSTVEKTVAPTECS

SEQ ID NO: 33 - protein, 288 aa, human
MQIPQAPWPVVWAVLQLGWRPGWFLDSPDRPWNPPTFSPALLVVTEGDNATFTCSFSNTSESFVLNWYRMSPSNQTDKLAAFPEDRSQPGQDCRFRVTQLPNGRDFHMSVVRARRNDSGTYLCGAISLAPKAQIKESLRAELRVTERRAEVPTAHPSPSPRPAGQFQTLVVGVVGGLLGSLVLLVWVLAVICSRAARGTIGARRTGQPLKEDPSAVPVFSVDYGELDFQWREKTPEPPVPCVPEQTEYATIVFPSGMGTSSPARRGSADGPRSAQPLRPEDGHCSWPL

SEQ ID NO: 34 - protein, 525 aa, human
MWEAQFLGLLFLQPLWVAPVKPLQPGAEVPVVWAQEGAPAQLPCSPTIPLQDLSLLRRAGVTWQHQPDSGPPAAAPGHPLAPGPHPAAPSSWGPRPRRYTVLSVGPGGLRSGRLPLQPRVQLDERGRQRGDFSLWLRPARRADAGEYRAAVHLRDRALSCRLRLRLGQASMTASPPGSLRASDWVILNCSFSRPDRPASVHWFRNRGQGRVPVRESPHHHLAESFLFLPQVSPMDSGPWGCILTYRDGFNVSIMYNLTVLGLEPPTPLTVYAGAGSRVGLPCRLPAGVGTRSFLTAKWTPPGGGPDLLVTGDNGDFTLRLEDVSQAQAGTYTCHIHLQEQQLNATVTLAIITVTPKSFGSPGSLGKLLCEVTPVSGQERFVWSSLDTPSQRSFSGPWLEAQEAQLLSQPWQCQLYQGERLLGAAVYFTELSSPGAQRSGRAPGALPAGHLLLFLILGVLSLLLLVTGAFGFHLWRRQWRPRRFSALEQGIHPPQAQSKIEELEQEPEPEPEPEPEPEPEPEPEQL

SEQ ID NO: 35 - RNA, 1378 nt, synthetic construct
  misc_feature 1..1378: note = mRNA corresponding to artificial DNA construct
  source 1..1378: mol_type = other RNA
gggagaaagcttaccatgggcagcatcggggccgcgtcgatggagttctgcttcgacgtgttcaaggagctgaaggtccaccacgccaacgagaacatcttctactgcccgatcgccatcatgagcgcgctcgccatggtgtacctgggcgccaaggacagcacccggacgcagatcaacaaggtggtccgcttcgacaagctgcccggcttcggggactcgatcgaggcgcagtgcggcaccagcgtgaacgtgcacagctcgctccgggacatcctgaaccagatcaccaagccgaacgacgtctacagcttcagcctggcctcgcggctctacgccgaggagcgctacccgatcctgcccgagtacctgcagtgcgtgaaggagctctaccggggcgggctggagccgatcaacttccagacggcggccgaccaggcccgggagctgatcaacagctgggtggagagccagaccaacggcatcatccgcaacgtcctccagccgtcgagcgtggacagccagaccgcgatggtgctggtcaacgccatcgtgttcaagggcctgtgggagaagacgttcaaggacgaggacacccaggccatgcccttccgggtgaccgagcaggagtcgaagccggtccagatgatgtaccagatcgggctcttccgggtggcgagcatggccagcgagaagatgaagatcctggagctgccgttcgcctcgggcacgatgagcatgctcgtgctgctgcccgacgaggtcagcggcctcgagcagctggagtcgatcatcaacttcgagaagctgaccgagtggaccagcagcaacgtgatggaggagcgcaagatcaaggtgtacctcccgcggatgaagatggaggagaagtacaacctgacgtcggtcctgatggcgatggggatcaccgacgtgttcagcagctcggccaacctcagcggcatcagctcggccgagagcctgaagatcagccaggcggtgcacgccgcccacgcggagatcaacgaggccggccgggaggtcgtggggtcggccgaggcgggcgtggacgccgccagcgtcagcgaggagttccgcgcggaccacccgttcctgttctgcatcaagcacatcgccaccaacgccgtgctcttcttcggccggtgcgtgtcgccctgaccactagttataagactgactagcccgatgggcctcccaacgggccctcctcccctccttgcaccgagattaataaaaaaaaaaaaaaaaaaaaaaaaaaaaaaaaaaaaaaaaaaaaaaaaaaaaaaaaaaaaaaaatgcatcccccccccccccccccccccccccccccccaaaggctcttttcagagccaccagaatt